European Patent Specification EP 4 001 303 B1, published May 7, 2025. Title: Novel method for preparing a long-acting drug conjugate using a intermediate. Applicant: HANMI PHARM. CO., LTD. The sequence listing filed with the application follows.

SEQUENCE LISTING (10 sequences)

SEQ ID NO: 1 - protein, 40 aa, Artificial Sequence
  GLP-1/GIP/Glucagon Triple Agonist analog 1
  VARIANT (2): Xaa = aminoisobutyric acid
YXQGTFTSDYSKYLDEKRAKEFVQWLLDHHPSSGQPPPSC

SEQ ID NO: 2 - protein, 39 aa, Artificial Sequence
  GLP-1/GIP/Glucagon Triple Agonist analog 2
  VARIANT (2): Xaa = aminoisobutyric acid
YXQGTFTSDYSKYLDEKRAKEFVQWLLDHHCSSGQPPPS

SEQ ID NO: 3 - protein, 40 aa, Artificial Sequence
  GLP-1/GIP/Glucagon Triple Agonist analog 3
  VARIANT (2): Xaa = aminoisobutyric acid
HXQGTFTSDYSKYLDEKRAKEFVQWLLDHHPSSGQPPPSC

SEQ ID NO: 4 - protein, 30 aa, Artificial Sequence
  Glucagon analog 1
  VARIANT (2): Xaa = aminoisobutyric acid
YXQGTFTSDYSKYLDEKRAKEFVQWLMNTC

SEQ ID NO: 5 - protein, 29 aa, Artificial Sequence
  Glucagon analog 2
  VARIANT (2): Xaa = aminoisobutyric acid
YXQGTFTSDYSKYLDECRAKEFVQWLMNT

SEQ ID NO: 6 - protein, 30 aa, Artificial Sequence
  Glucagon analog 3
  VARIANT (2): Xaa = aminoisobutyric acid
YXQGTFTSDYSKYLDSRRAQDFVQWLMNTC

SEQ ID NO: 7 - protein, 12 aa, homo sapiens
ESKYGPPCPSCP

SEQ ID NO: 8 - protein, 3 aa, Artificial Sequence
  Variant of hinge region
SCP

SEQ ID NO: 9 - protein, 4 aa, Artificial Sequence
  Variant of hinge region
PSCP

SEQ ID NO: 10 - protein, 221 aa, homo sapiens
PSCPAPEFLGGPSVFLFPPKPKDTLMISRTPEVTCVVVDVSQEDPEVQFNWYVDGVEVHNAKTKPREEQFNSTYRVVSVLTVLHQDWLNGKEYKCKVSNKGLPSSIEKTISKAKGQPREPQVYTLPPSQEEMTKNQVSLTCLVKGFYPSDIAVEWESNGQPENNYKTTPPVLDSDGSFFLYSRLTVDKSRWQEGNVFSCSVMHEALHNHYTQKSLSLSLGK